European Patent Application EP 4 741 418 A1, published May 13, 2026. Title: 一种角蛋白CF1、制法和其药物组合物与用途. Applicant: 中国医学科学院药物研究所. The sequence listing filed with the application follows.

SEQUENCE LISTING (2 sequences)

SEQ ID NO: 1 - protein, 585 aa, unidentified
MSCRSYRVSSGHRVGNFSSCSAGIPRNLNRFRASSVSCRSGPSFRGIGGFGSRSVITFGSCSPRIAAVGPRPIRCGVGFGAGSGMAFGFGDGIGAGLGFGSGSYLGYGFGGPGFGYRVGGIGVPAAPSITPVTVNQSLLTPLNLEIDPNAQRVKRDEKEQIKTLNNRFASFIDKVRFLEQQNKLLETKWSFLQEQKGARSNLEPLFENYITNLQRQLDIANSERARFEAERNQLQDVLEGFKKKYEEEVVFRANAENEFVALKKDVDAAFLNKAELEANVDTLTQEIDFLKTLYAAEIQLLQSHISETSVIVKMDNSRDLDLDGIIAEVRAQYEEVAKRSRADAEAWYQTKYEEMRVTAGQHCDNLRNTREEINELTRLIQRLKAEIEHAKAQRARLEAAVAEAEQQGEAALNDAKCKLADLEAALQQAKQDMARQLREYQELMNAKLGLDIEIATYRRLLEGEEIRICEGVGPVNISVSSSRGGVVCGPESLVTSSTLSRSGVTFSGSSSIRPSGACGSSLGGVVVAGGDLLSAGSRGGSVLVGEACVPSVPCPLPTEGFSSCSGGRSSSLRFVSTTTSRRTKY

SEQ ID NO: 2 - DNA, 1755 bp, unidentified
  source 1..1755: mol_type = other DNA
atgagctgccgcagctatcgcgtgagcagcggccatcgtgttggcaactttagcagctgcagcgcgggcattccgcgcaatttaaaccgctttcgcgcgagcagcgtgagctgccgtagcggacctagctttcgtggtattggtggctttggcagccgcagcgtgattacctttggcagctgcagcccgcgcattgcggcggttggtcctcgtcctattcgttgtggtgtgggctttggcgcgggtagcggtatggcgtttggttttggcgatggcattggcgcgggcctgggttttggtagcggtagctatttaggttatggctttggcggcccgggctttggctatcgcgttggtggtattggcgtgccggcggcgcctagcattacccctgttaccgttaatcagagcctgctgaccccgctgaacctggaaattgatccgaacgcgcagcgcgtgaaacgcgatgaaaaagaacagattaaaaccctgaacaaccgctttgcgagctttattgataaagtgcgctttctggaacagcagaacaaactgctggaaaccaaatggagctttctgcaggaacagaaaggcgcccgtagcaacctggaaccgctgtttgaaaactatattaccaacctgcagcgccagctggatattgcgaacagcgaacgcgcacgctttgaagcggaacgcaatcagctgcaggatgtgctggaaggctttaaaaagaaatatgaggaggaggtggtgttccgcgcgaacgcggaaaatgaatttgtggcgctgaaaaaggatgtggatgcggcgtttctgaacaaagcggaactggaagcgaacgtggataccctgacccaggaaattgattttctgaaaaccctgtatgcggcggaaattcagctgctgcagagccatattagcgaaaccagcgtgattgtgaaaatggataacagccgcgatctggatctggatggcattattgcggaagtgcgtgcgcaatatgaagaagtggcgaaacgcagccgcgcggatgcggaagcatggtatcaaaccaaatatgaagaaatgcgcgtgaccgcgggccagcattgcgataatctgcgcaacacccgcgaagaaattaacgaactgacccgcctgattcagcgcctgaaagcggaaattgaacatgcgaaagcgcaacgcgcacgcctggaagcggcggtggcggaagcggaacaacaaggtgaagcggcgctgaacgatgcgaaatgcaaactggcggatctggaagcggcgctgcagcaggcgaaacaggatatggcccgccagctgcgcgaatatcaggaactgatgaacgcgaaactgggcctggatattgaaattgcgacctatcgccgcctgctggaaggcgaagaaattcgcatttgcgaaggcgtgggcccggtgaacattagcgtgagctcaagccgcggcggcgttgtttgtggtcctgaatcgttagtgaccagcagcaccctgagccgcagcggtgttacctttagcggcagctcaagcattcgcccgagcggcgcgtgtggtagcagcttaggtggtgttgttgttgcgggcggtgatctgctgagcgcgggtagccgtggtggttcagttttggttggcgaagcgtgcgtgcctagcgttccgtgtcctttacctaccgaaggttttagcagctgcagcggcggccgctcaagcagcttacgttttgtgagcaccaccaccagccgccgcaccaaatat